European Patent Application EP 4 148 065 A1, published March 15, 2023. Title: Chimera antigen receptors for treating cancer. Applicant: SMT bio Industry-Academic Cooperation Foundation, Yonsei University. The sequence listing filed with the application follows.

SEQUENCE LISTING (20 sequences)

SEQ ID NO: 1 - protein, 111 aa, Artificial Sequence
  VH domain
DIVLTQSPASLAVSLGQRATMSCRAGESVDIFGVGFLHWYQQKPGQPPKLLIYRASNLESGIPVRFSGTGSRTDFTLIIDPVEADDVATYYCQQTNEDPYTFGGGTKLEIK

SEQ ID NO: 2 - protein, 121 aa, Artificial Sequence
  VL domain
EVQLQQSGAELVEPGASVKLSCTASGFNIKDTYMHWVKQRPEQGLEWIGRIDPANGNSKYVPKFQGKATITADTSSNTAYLQLTSLTSEDTAVYYCAPFGYYVSDYAMAYWGQGTSVTVSS

SEQ ID NO: 3 - protein, 15 aa, Artificial Sequence
  linker
GGGGSGGGGSGGGGS

SEQ ID NO: 4 - protein, 45 aa, Artificial Sequence
  hinge region
TTTPAPRPPTPAPTIASQPLSLRPEACRPAAGGAVHTRGLDFACD

SEQ ID NO: 5 - protein, 24 aa, Artificial Sequence
  transmembrane domain
IYIWAPLAGTCGVLLLSLVITLYC

SEQ ID NO: 6 - protein, 42 aa, Artificial Sequence
  co-stimulatory domain
KRGRKKLLYIFKQPFMRPVQTTQEEDGCSCRFPEEEEGGCEL

SEQ ID NO: 7 - protein, 112 aa, Artificial Sequence
  signal transduction domain
RVKFSRSADAPAYKQGQNQLYNELNLGRREEYDVLDKRRGRDPEMGGKPRRKNPQEGLYNELQKDKMAEAYSEIGMKGERRRGKGHDGLYQGLSTATKDTYDALHMQALPPR

SEQ ID NO: 8 - protein, 21 aa, Artificial Sequence
  signal peptide
MALPVTALLLPLALLLHAARP

SEQ ID NO: 9 - protein, 470 aa, Artificial Sequence
  chimeric antigen receptor
DIVLTQSPASLAVSLGQRATMSCRAGESVDIFGVGFLHWYQQKPGQPPKLLIYRASNLESGIPVRFSGTGSRTDFTLIIDPVEADDVATYYCQQTNEDPYTFGGGTKLEIKGGGGSGGGGSGGGGSEVQLQQSGAELVEPGASVKLSCTASGFNIKDTYMHWVKQRPEQGLEWIGRIDPANGNSKYVPKFQGKATITADTSSNTAYLQLTSLTSEDTAVYYCAPFGYYVSDYAMAYWGQGTSVTVSSTTTPAPRPPTPAPTIASQPLSLRPEACRPAAGGAVHTRGLDFACDIYIWAPLAGTCGVLLLSLVITLYCKRGRKKLLYIFKQPFMRPVQTTQEEDGCSCRFPEEEEGGCELRVKFSRSADAPAYKQGQNQLYNELNLGRREEYDVLDKRRGRDPEMGGKPRRKNPQEGLYNELQKDKMAEAYSEIGMKGERRRGKGHDGLYQGLSTATKDTYDALHMQALPPR

SEQ ID NO: 10 - protein, 491 aa, Artificial Sequence
  chimeric antigen receptor
MALPVTALLLPLALLLHAARPDIVLTQSPASLAVSLGQRATMSCRAGESVDIFGVGFLHWYQQKPGQPPKLLIYRASNLESGIPVRFSGTGSRTDFTLIIDPVEADDVATYYCQQTNEDPYTFGGGTKLEIKGGGGSGGGGSGGGGSEVQLQQSGAELVEPGASVKLSCTASGFNIKDTYMHWVKQRPEQGLEWIGRIDPANGNSKYVPKFQGKATITADTSSNTAYLQLTSLTSEDTAVYYCAPFGYYVSDYAMAYWGQGTSVTVSSTTTPAPRPPTPAPTIASQPLSLRPEACRPAAGGAVHTRGLDFACDIYIWAPLAGTCGVLLLSLVITLYCKRGRKKLLYIFKQPFMRPVQTTQEEDGCSCRFPEEEEGGCELRVKFSRSADAPAYKQGQNQLYNELNLGRREEYDVLDKRRGRDPEMGGKPRRKNPQEGLYNELQKDKMAEAYSEIGMKGERRRGKGHDGLYQGLSTATKDTYDALHMQALPPR

SEQ ID NO: 11 - DNA, 1410 bp, Artificial Sequence
  chimeric antigen receptor
gacatcgtgctgacacagagccctgcttctctggccgtgtctcttggacagagggccaccatgtcttgtagagccggcgagagcgtggacatcttcggcgtgggatttctgcactggtatcagcagaagcccggccagcctcctaagctgctgatctacagagccagcaacctggaaagcggcatccctgtgcggtttagcggcacaggcagcagaaccgacttcaccctgatcatcgaccccgtggaagccgatgatgtggccacctactactgccagcagaccaacgaggacccctacacatttggcggaggcaccaagctggaaatcaagggtggaggtggcagcggaggaggtgggtccggcggtggaggaagcgaggttcagctgcagcagtctggcgctgaactggttgaacctggcgcctctgtgaagctgagctgtaccgccagcggcttcaacatcaaggacacctacatgcactgggtcaagcagaggcctgagcagggactcgagtggatcggcagaatcgatcccgccaacggcaacagcaaatacgtgcccaagttccagggcaaagccaccatcaccgccgacacctctagcaacacagcctacctgcagctcaccagcctgacctctgaagataccgccgtgtactactgcgcccctttcggctactacgtgtccgattacgccatggcctattggggccagggcacaagcgtgacagtcagctctaccacgacgccagcgccgcgaccaccaacaccggcgcccaccatcgcgtcgcagcccctgtccctgcgcccagaggcgtgccggccagcggcggggggcgcagtgcacacgagggggctggacttcgcctgtgatatctacatttgggcccctctggctggtacttgcggggtcctgctgctttcactcgtgatcactctttactgtaagcgcggtcggaagaagctgctgtacatctttaagcaacccttcatgaggcctgtgcagactactcaagaggaggacggctgttcatgccggttcccagaggaggaggaaggcggctgcgaactgagagtgaagttcagcaggagcgcagacgcccccgcgtacaagcagggccagaaccagctctataacgagctcaatctaggacgaagagaggagtacgatgttttggacaagagacgtggccgggaccctgagatggggggaaagccgagaaggaagaaccctcaggaaggcctgtacaatgaactgcagaaagataagatggcggaggcctacagtgagattgggatgaaaggcgagcgccggaggggcaaggggcacgatggcctttaccagggtctcagtacagccaccaaggacacctacgacgcccttcacatgcaggccctgccccctcgc

SEQ ID NO: 12 - DNA, 1473 bp, Artificial Sequence
  chimeric antigen receptor
atggccttaccagtgaccgccttgctcctgccgctggccttgctgctccacgccgccaggccggacatcgtgctgacacagagccctgcttctctggccgtgtctcttggacagagggccaccatgtcttgtagagccggcgagagcgtggacatcttcggcgtgggatttctgcactggtatcagcagaagcccggccagcctcctaagctgctgatctacagagccagcaacctggaaagcggcatccctgtgcggtttagcggcacaggcagcagaaccgacttcaccctgatcatcgaccccgtggaagccgatgatgtggccacctactactgccagcagaccaacgaggacccctacacatttggcggaggcaccaagctggaaatcaagggtggaggtggcagcggaggaggtgggtccggcggtggaggaagcgaggttcagctgcagcagtctggcgctgaactggttgaacctggcgcctctgtgaagctgagctgtaccgccagcggcttcaacatcaaggacacctacatgcactgggtcaagcagaggcctgagcagggactcgagtggatcggcagaatcgatcccgccaacggcaacagcaaatacgtgcccaagttccagggcaaagccaccatcaccgccgacacctctagcaacacagcctacctgcagctcaccagcctgacctctgaagataccgccgtgtactactgcgcccctttcggctactacgtgtccgattacgccatggcctattggggccagggcacaagcgtgacagtcagctctaccacgacgccagcgccgcgaccaccaacaccggcgcccaccatcgcgtcgcagcccctgtccctgcgcccagaggcgtgccggccagcggcggggggcgcagtgcacacgagggggctggacttcgcctgtgatatctacatttgggcccctctggctggtacttgcggggtcctgctgctttcactcgtgatcactctttactgtaagcgcggtcggaagaagctgctgtacatctttaagcaacccttcatgaggcctgtgcagactactcaagaggaggacggctgttcatgccggttcccagaggaggaggaaggcggctgcgaactgagagtgaagttcagcaggagcgcagacgcccccgcgtacaagcagggccagaaccagctctataacgagctcaatctaggacgaagagaggagtacgatgttttggacaagagacgtggccgggaccctgagatggggggaaagccgagaaggaagaaccctcaggaaggcctgtacaatgaactgcagaaagataagatggcggaggcctacagtgagattgggatgaaaggcgagcgccggaggggcaaggggcacgatggcctttaccagggtctcagtacagccaccaaggacacctacgacgcccttcacatgcaggccctgccccctcgc

SEQ ID NO: 13 - protein, 352 aa, Artificial Sequence
  EGFRt
MWLQSLLLLGTVACSISRKVCNGIGIGEFKDSLSINATNIKHFKNCTSISGDLHILPVAFRGDSFTHTPPLDPQELDILKTVKEITGFLLIQAWPENRTDLHAFENLEIIRGRTKQHGQFSLAVVSLNITSLGLRSLKEISDGDVIISGNKNLCYANTINWKKLFGTSGQKTKIISNRGENSCKATGQVCHALCSPEGCWGPEPRDCVSCRNVSRGRECVDKCNLLEGEPREFVENSECIQCHPECLPQAMNITCTGRGPDNCIQCAHYIDGPHCVKTCPAGVMGENNTLVWKYADAGHVCHLCHPNCTYGCTGPGLEGCPTNGPKIPSIATGMVGALLLLLVVALGIGLFM

SEQ ID NO: 14 - DNA, 1056 bp, Artificial Sequence
  EGFRt
atgtggctgcagagcctgctgctcttgggcactgtggcctgcagcatctctcgcaaagtgtgtaacggaataggtattggtgaatttaaagactcactctccataaatgctacgaatattaaacacttcaaaaactgcacctccatcagtggcgatctccacatcctgccggtggcatttaggggtgactccttcacacatactcctcctctggatccacaggaactggatattctgaaaaccgtaaaggaaatcacagggtttttgctgattcaggcttggcctgaaaacaggacggacctccatgcctttgagaacctagaaatcatacgcggcaggaccaagcaacatggtcagttttctcttgcagtcgtcagcctgaacataacatccttgggattacgctccctcaaggagataagtgatggagatgtgataatttcaggaaacaaaaatttgtgctatgcaaatacaataaactggaaaaaactgtttgggacctccggtcagaaaaccaaaattataagcaacagaggtgaaaacagctgcaaggccacaggccaggtctgccatgccttgtgctcccccgagggctgctggggcccggagcccagggactgcgtctcttgccggaatgtcagccgaggcagggaatgcgtggacaagtgcaaccttctggagggtgagccaagggagtttgtggagaactctgagtgcatacagtgccacccagagtgcctgcctcaggccatgaacatcacctgcacaggacggggaccagacaactgtatccagtgtgcccactacattgacggcccccactgcgtcaagacctgcccggcaggagtcatgggagaaaacaacaccctggtctggaagtacgcagacgccggccatgtgtgccacctgtgccatccaaactgcacctacggatgcactgggccaggtcttgaaggctgtccaacgaatgggcctaagatcccgtccatcgccactgggatggtgggggccctcctcttgctgctggtggtggccctggggatcggcctcttcatg

SEQ ID NO: 15 - protein, 18 aa, Artificial Sequence
  T2A
EGRGSLLTCGDVEENPGP

SEQ ID NO: 16 - DNA, 54 bp, Artificial Sequence
  T2A
gagggcaggggaagtcttctaacatgcggggacgtggaggaaaatcccggcccc

SEQ ID NO: 17 - DNA, 2880 bp, Artificial Sequence
  chimeric antigen receptor cassette
gagtaattcatacaaaaggactcgcccctgccttggggaatcccagggaccgtcgttaaactcccactaacgtagaacccagagatcgctgcgttcccgccccctcacccgcccgctctcgtcatcactgaggtggagaagagcatgcgtgaggctccggtgcccgtcagtgggcagagcgcacatcgcccacagtccccgagaagttggggggaggggtcggcaattgaaccggtgcctagagaaggtggcgcggggtaaactgggaaagtgatgtcgtgtactggctccgcctttttcccgagggtgggggagaaccgtatataagtgcagtagtcgccgtgaacgttctttttcgcaacgggtttgccgccagaacacaggtaagtgccgtgtgtggttcccgcgggcctggcctctttacgggttatggcccttgcgtgccttgaattacttccacgcccctggctgcagtacgtgattcttgatcccgagcttcgggttggaagtgggtgggagagttcgaggccttgcgcttaaggagccccttcgcctcgtgcttgagttgaggcctggcttgggcgctggggccgccgcgtgcgaatctggtggcaccttcgcgcctgtctcgctgctttcgataagtctctagccatttaaaatttttgatgacctgctgcgacgctttttttctggcaagatagtcttgtaaatgcgggccaagatctgcacactggtatttcggtttttggggccgcgggcggcgacggggcccgtgcgtcccagcgcacatgttcggcgaggcggggcctgcgagcgcggccaccgagaatcggacgggggtagtctcaagctggccggcctgctctggtgcctggcctcgcgccgccgtgtatcgccccgccctgggcggcaaggctggcccggtcggcaccagttgcgtgagcggaaagatggccgcttcccggccctgctgcagggagctcaaaatggaggacgcggcgctcgggagagcgggcgggtgagtcacccacacaaaggaaaagggcctttccgtcctcagccgtcgcttcatgtgactccacggagtaccgggcgccgtccaggcacctcgattagttctcgagcttttggagtacgtcgtctttaggttggggggaggggttttatgcgatggagtttccccacactgagtgggtggagactgaagttaggccagcttggcacttgatgtaattctccttggaatttgccctttttgagtttggatcttggttcattctcaagcctcagacagtggttcaaagtttttttcttccatttcaggtgtcgtgattcgaattcgccgccaccatggccttaccagtgaccgccttgctcctgccgctggccttgctgctccacgccgccaggccggacatcgtgctgacacagagccctgcttctctggccgtgtctcttggacagagggccaccatgtcttgtagagccggcgagagcgtggacatcttcggcgtgggatttctgcactggtatcagcagaagcccggccagcctcctaagctgctgatctacagagccagcaacctggaaagcggcatccctgtgcggtttagcggcacaggcagcagaaccgacttcaccctgatcatcgaccccgtggaagccgatgatgtggccacctactactgccagcagaccaacgaggacccctacacatttggcggaggcaccaagctggaaatcaagggtggaggtggcagcggaggaggtgggtccggcggtggaggaagcgaggttcagctgcagcagtctggcgctgaactggttgaacctggcgcctctgtgaagctgagctgtaccgccagcggcttcaacatcaaggacacctacatgcactgggtcaagcagaggcctgagcagggactcgagtggatcggcagaatcgatcccgccaacggcaacagcaaatacgtgcccaagttccagggcaaagccaccatcaccgccgacacctctagcaacacagcctacctgcagctcaccagcctgacctctgaagataccgccgtgtactactgcgcccctttcggctactacgtgtccgattacgccatggcctattggggccagggcacaagcgtgacagtcagctctaccacgacgccagcgccgcgaccaccaacaccggcgcccaccatcgcgtcgcagcccctgtccctgcgcccagaggcgtgccggccagcggcggggggcgcagtgcacacgagggggctggacttcgcctgtgatatctacatttgggcccctctggctggtacttgcggggtcctgctgctttcactcgtgatcactctttactgtaagcgcggtcggaagaagctgctgtacatctttaagcaacccttcatgaggcctgtgcagactactcaagaggaggacggctgttcatgccggttcccagaggaggaggaaggcggctgcgaactgagagtgaagttcagcaggagcgcagacgcccccgcgtacaagcagggccagaaccagctctataacgagctcaatctaggacgaagagaggagtacgatgttttggacaagagacgtggccgggaccctgagatggggggaaagccgagaaggaagaaccctcaggaaggcctgtacaatgaactgcagaaagataagatggcggaggcctacagtgagattgggatgaaaggcgagcgccggaggggcaaggggcacgatggcctttaccagggtctcagtacagccaccaaggacacctacgacgcccttcacatgcaggccctgccccctcgcgagggcaggggaagtcttctaacatgcggggacgtggaggaaaatcccggcccc

SEQ ID NO: 18 - DNA, 3939 bp, Artificial Sequence
  chimeric antigen receptor cassette
gagtaattcatacaaaaggactcgcccctgccttggggaatcccagggaccgtcgttaaactcccactaacgtagaacccagagatcgctgcgttcccgccccctcacccgcccgctctcgtcatcactgaggtggagaagagcatgcgtgaggctccggtgcccgtcagtgggcagagcgcacatcgcccacagtccccgagaagttggggggaggggtcggcaattgaaccggtgcctagagaaggtggcgcggggtaaactgggaaagtgatgtcgtgtactggctccgcctttttcccgagggtgggggagaaccgtatataagtgcagtagtcgccgtgaacgttctttttcgcaacgggtttgccgccagaacacaggtaagtgccgtgtgtggttcccgcgggcctggcctctttacgggttatggcccttgcgtgccttgaattacttccacgcccctggctgcagtacgtgattcttgatcccgagcttcgggttggaagtgggtgggagagttcgaggccttgcgcttaaggagccccttcgcctcgtgcttgagttgaggcctggcttgggcgctggggccgccgcgtgcgaatctggtggcaccttcgcgcctgtctcgctgctttcgataagtctctagccatttaaaatttttgatgacctgctgcgacgctttttttctggcaagatagtcttgtaaatgcgggccaagatctgcacactggtatttcggtttttggggccgcgggcggcgacggggcccgtgcgtcccagcgcacatgttcggcgaggcggggcctgcgagcgcggccaccgagaatcggacgggggtagtctcaagctggccggcctgctctggtgcctggcctcgcgccgccgtgtatcgccccgccctgggcggcaaggctggcccggtcggcaccagttgcgtgagcggaaagatggccgcttcccggccctgctgcagggagctcaaaatggaggacgcggcgctcgggagagcgggcgggtgagtcacccacacaaaggaaaagggcctttccgtcctcagccgtcgcttcatgtgactccacggagtaccgggcgccgtccaggcacctcgattagttctcgagcttttggagtacgtcgtctttaggttggggggaggggttttatgcgatggagtttccccacactgagtgggtggagactgaagttaggccagcttggcacttgatgtaattctccttggaatttgccctttttgagtttggatcttggttcattctcaagcctcagacagtggttcaaagtttttttcttccatttcaggtgtcgtgattcgaattcgccgccaccatggccttaccagtgaccgccttgctcctgccgctggccttgctgctccacgccgccaggccggacatcgtgctgacacagagccctgcttctctggccgtgtctcttggacagagggccaccatgtcttgtagagccggcgagagcgtggacatcttcggcgtgggatttctgcactggtatcagcagaagcccggccagcctcctaagctgctgatctacagagccagcaacctggaaagcggcatccctgtgcggtttagcggcacaggcagcagaaccgacttcaccctgatcatcgaccccgtggaagccgatgatgtggccacctactactgccagcagaccaacgaggacccctacacatttggcggaggcaccaagctggaaatcaagggtggaggtggcagcggaggaggtgggtccggcggtggaggaagcgaggttcagctgcagcagtctggcgctgaactggttgaacctggcgcctctgtgaagctgagctgtaccgccagcggcttcaacatcaaggacacctacatgcactgggtcaagcagaggcctgagcagggactcgagtggatcggcagaatcgatcccgccaacggcaacagcaaatacgtgcccaagttccagggcaaagccaccatcaccgccgacacctctagcaacacagcctacctgcagctcaccagcctgacctctgaagataccgccgtgtactactgcgcccctttcggctactacgtgtccgattacgccatggcctattggggccagggcacaagcgtgacagtcagctctaccacgacgccagcgccgcgaccaccaacaccggcgcccaccatcgcgtcgcagcccctgtccctgcgcccagaggcgtgccggccagcggcggggggcgcagtgcacacgagggggctggacttcgcctgtgatatctacatttgggcccctctggctggtacttgcggggtcctgctgctttcactcgtgatcactctttactgtaagcgcggtcggaagaagctgctgtacatctttaagcaacccttcatgaggcctgtgcagactactcaagaggaggacggctgttcatgccggttcccagaggaggaggaaggcggctgcgaactgagagtgaagttcagcaggagcgcagacgcccccgcgtacaagcagggccagaaccagctctataacgagctcaatctaggacgaagagaggagtacgatgttttggacaagagacgtggccgggaccctgagatggggggaaagccgagaaggaagaaccctcaggaaggcctgtacaatgaactgcagaaagataagatggcggaggcctacagtgagattgggatgaaaggcgagcgccggaggggcaaggggcacgatggcctttaccagggtctcagtacagccaccaaggacacctacgacgcccttcacatgcaggccctgccccctcgcgagggcaggggaagtcttctaacatgcggggacgtggaggaaaatcccggccccatgtggctgcagagcctgctgctcttgggcactgtggcctgcagcatctctcgcaaagtgtgtaacggaataggtattggtgaatttaaagactcactctccataaatgctacgaatattaaacacttcaaaaactgcacctccatcagtggcgatctccacatcctgccggtggcatttaggggtgactccttcacacatactcctcctctggatccacaggaactggatattctgaaaaccgtaaaggaaatcacagggtttttgctgattcaggcttggcctgaaaacaggacggacctccatgcctttgagaacctagaaatcatacgcggcaggaccaagcaacatggtcagttttctcttgcagtcgtcagcctgaacataacatccttgggattacgctccctcaaggagataagtgatggagatgtgataatttcaggaaacaaaaatttgtgctatgcaaatacaataaactggaaaaaactgtttgggacctccggtcagaaaaccaaaattataagcaacagaggtgaaaacagctgcaaggccacaggccaggtctgccatgccttgtgctcccccgagggctgctggggcccggagcccagggactgcgtctcttgccggaatgtcagccgaggcagggaatgcgtggacaagtgcaaccttctggagggtgagccaagggagtttgtggagaactctgagtgcatacagtgccacccagagtgcctgcctcaggccatgaacatcacctgcacaggacggggaccagacaactgtatccagtgtgcccactacattgacggcccccactgcgtcaagacctgcccggcaggagtcatgggagaaaacaacaccctggtctggaagtacgcagacgccggccatgtgtgccacctgtgccatccaaactgcacctacggatgcactgggccaggtcttgaaggctgtccaacgaatgggcctaagatcccgtccatcgccactgggatggtgggggccctcctcttgctgctggtggtggccctggggatcggcctcttcatgtaa

SEQ ID NO: 19 - protein, 840 aa, Artificial Sequence
  synthetic sequence
DIVLTQSPASLAVSLGQRATMSCRAGESVDIFGVGFLHWYQQKPGQPPKLLIYRASNLESGIPVRFSGTGSRTDFTLIIDPVEADDVATYYCQQTNEDPYTFGGGTKLEIKGGGGSGGGGSGGGGSEVQLQQSGAELVEPGASVKLSCTASGFNIKDTYMHWVKQRPEQGLEWIGRIDPANGNSKYVPKFQGKATITADTSSNTAYLQLTSLTSEDTAVYYCAPFGYYVSDYAMAYWGQGTSVTVSSTTTPAPRPPTPAPTIASQPLSLRPEACRPAAGGAVHTRGLDFACDIYIWAPLAGTCGVLLLSLVITLYCKRGRKKLLYIFKQPFMRPVQTTQEEDGCSCRFPEEEEGGCELRVKFSRSADAPAYKQGQNQLYNELNLGRREEYDVLDKRRGRDPEMGGKPRRKNPQEGLYNELQKDKMAEAYSEIGMKGERRRGKGHDGLYQGLSTATKDTYDALHMQALPPREGRGSLLTCGDVEENPGPMWLQSLLLLGTVACSISRKVCNGIGIGEFKDSLSINATNIKHFKNCTSISGDLHILPVAFRGDSFTHTPPLDPQELDILKTVKEITGFLLIQAWPENRTDLHAFENLEIIRGRTKQHGQFSLAVVSLNITSLGLRSLKEISDGDVIISGNKNLCYANTINWKKLFGTSGQKTKIISNRGENSCKATGQVCHALCSPEGCWGPEPRDCVSCRNVSRGRECVDKCNLLEGEPREFVENSECIQCHPECLPQAMNITCTGRGPDNCIQCAHYIDGPHCVKTCPAGVMGENNTLVWKYADAGHVCHLCHPNCTYGCTGPGLEGCPTNGPKIPSIATGMVGALLLLLVVALGIGLFM

SEQ ID NO: 20 - protein, 861 aa, Artificial Sequence
  synthetic sequence
MALPVTALLLPLALLLHAARPDIVLTQSPASLAVSLGQRATMSCRAGESVDIFGVGFLHWYQQKPGQPPKLLIYRASNLESGIPVRFSGTGSRTDFTLIIDPVEADDVATYYCQQTNEDPYTFGGGTKLEIKGGGGSGGGGSGGGGSEVQLQQSGAELVEPGASVKLSCTASGFNIKDTYMHWVKQRPEQGLEWIGRIDPANGNSKYVPKFQGKATITADTSSNTAYLQLTSLTSEDTAVYYCAPFGYYVSDYAMAYWGQGTSVTVSSTTTPAPRPPTPAPTIASQPLSLRPEACRPAAGGAVHTRGLDFACDIYIWAPLAGTCGVLLLSLVITLYCKRGRKKLLYIFKQPFMRPVQTTQEEDGCSCRFPEEEEGGCELRVKFSRSADAPAYKQGQNQLYNELNLGRREEYDVLDKRRGRDPEMGGKPRRKNPQEGLYNELQKDKMAEAYSEIGMKGERRRGKGHDGLYQGLSTATKDTYDALHMQALPPREGRGSLLTCGDVEENPGPMWLQSLLLLGTVACSISRKVCNGIGIGEFKDSLSINATNIKHFKNCTSISGDLHILPVAFRGDSFTHTPPLDPQELDILKTVKEITGFLLIQAWPENRTDLHAFENLEIIRGRTKQHGQFSLAVVSLNITSLGLRSLKEISDGDVIISGNKNLCYANTINWKKLFGTSGQKTKIISNRGENSCKATGQVCHALCSPEGCWGPEPRDCVSCRNVSRGRECVDKCNLLEGEPREFVENSECIQCHPECLPQAMNITCTGRGPDNCIQCAHYIDGPHCVKTCPAGVMGENNTLVWKYADAGHVCHLCHPNCTYGCTGPGLEGCPTNGPKIPSIATGMVGALLLLLVVALGIGLFM